European Patent Application EP 4 317 447 A2, published February 7, 2024. Title: DONOR REPAIR TEMPLATES MULTIPLEX GENOME EDITING. Applicant: 2seventy bio, Inc. The sequence listing filed with the application follows.

SEQUENCE LISTING (40 sequences)

SEQ ID NO: 1 - DNA, 7317 bp, synthetic construct
  misc_feature 1..7317: note = Synthesized sequence pBW1411
  source 1..7317: mol_type = other DNA
cagctgcgcgctcgctcgctcactgaggccgcccgggcaaagcccgggcgtcgggcgacctttggtcgcccggcctcagtgagcgagcgagcgcgcagagagggagtggccaactccatcactaggggttccttgtagttaatgattaacccgccatgctacttatctacgtaaggctgttgcaggcatcacacggtggaaagatctggaactgtggccatggtgtgaggccatccacaaggtggaagctttgagggggagccgattagccatggacagttgtcattcagtagggtcacctgtgccccagcgaagggggatgggccgggaaggcagaggccaggcacctgcccccagcaggggcagaggctgtgggcagccgggaggctcccagaggctccgacagaatgggagtggggttgagcccacccctcactgcagcccaggaacctgagcccagagggggccacccaccttccccaggcagggaggcccggcccccagggagatgggggggatgggggaggagaagggcctgcccccacccggcagcctcaggaggggcagctcgggcgggatatggaaagaggccacagcagtgagcagagacacagaggaggaaggggccctgagctggggagacccccacggggtagggcgtgggggccacgggcccacctcctccccatctcctctgtctccctgtctctgtctctctctccctcccccaccctctccccagtcctaccccctcctcacccctcctcccccagcactgcctctgtcactctcgcccacgtggatgtggaggaagagggggcgggagcaaggggcgggcaccctcccttcaacctgacctgggacagtttcccttccgctcacctccgcctgagcagtggagaaggcggcactctggtggggctgctccaaatcatggcctcttggccaagattgatagcttgtgcctgtccctgagtcccagtccatcacgagcagctggtttctaagatgctatttcccgtataaagcatgagaccgtgacttgccagccccacagagccccgcccttgtccatcactggcatctggactccagcctgggttggggcaaagagggaaatgagatcatgtcctaaccctgatcctcttgtcccacagatatccagaaccctgaccctgccgtgtaccagctgagagactctaaatccagtgacaagtctgtctgcctatcgcgtgaacagagaaacaggagaatatgggccaaacaggatatctgtggtaagcagttcctgccccggctcagggccaagaacagttggaacagcagaatatgggccaaacaggatatctgtggtaagcagttcctgccccggctcagggccaagaacagatggtccccagatgcggtcccgccctcagcagtttctagagaaccatcagatgtttccagggtgccccaaggacctgaaatgaccctgtgccttatttgaactaaccaatcagttcgcttctcgcttctgttcgcgcgcttctgctccccgagctctatataagcagagctcgtttagtgaaccgtcagatcgcctggagacgccatccacgctgttttgacttccatagaaggatctcgaggccaccatggtgagcaagggcgaggagctgttcaccggggtggtgcccatcctggtcgagctggacggcgacgtaaacggccacaagttcagcgtgtccggcgagggcgagggcgatgccacctacggcaagctgaccctgaagttcatctgcaccaccggcaagctgcccgtgccctggcccaccctcgtgaccaccctgacctacggcgtgcagtgcttcagccgctaccccgaccacatgaagcagcacgacttcttcaagtccgccatgcccgaaggctacgtccaggagcgcaccatcttcttcaaggacgacggcaactacaagacccgcgccgaggtgaagttcgagggcgacaccctggtgaaccgcatcgagctgaagggcatcgacttcaaggaggacggcaacatcctggggcacaagctggagtacaactacaacagccacaacgtctatatcatggccgacaagcagaagaacggcatcaaggtgaacttcaagatccgccacaacatcgaggacggcagcgtgcagctcgccgaccactaccagcagaacacccccatcggcgacggccccgtgctgctgcccgacaaccactacctgagcacccagtccgccctgagcaaagaccccaacgagaagcgcgatcacatggtcctgctggagttcgtgaccgccgccgggatcactctcggcatggacgagctgtacaagtaagcggccgcgctttatttgtgaaatttgtgatgctattgctttatttgtaaccattataagctgcaataaacaagttaacaacaacaattgcattcattttatgtttcaggttcagggggagatgtgggaggttttttaaagcctctttgattctcaaacaaatgtgtcacaaagtaaggattctgatgtgtatatcacagacaaaactgtgctagacatgaggtctatggacttcaagagcaacagtgctgtggcctggagcaacaaatctgactttgcatgtgcaaacgccttcaacaacagcattattccagaagacaccttcttccccagcccaggtaagggcagctttggtgccttcgcaggctgtttccttgcttcaggaatggccaggttctgcccagagctctggtcaatgatgtctaaaactcctctgattggtggtaccggttctgggcggtgctacaactgggctggcggccaggatggttcttaggtaggtggggtcggcggtcaggtgtcccagagccaggggtctggagggaccttccaccctcagtccctggcaggtcggggggtgctgaggcgggcctggccctggcagcccaggggtcccggagcgaggggtctggagggacctttcactctcagtccctggcaggtcggggggtgctgtggcaggcccagccttggcccccagctctgccccttaccctgagctgtgtggctttgggcagctcgaactcctgggttcctctctgggccccaactcctcccctggcccaagtcccctctttgctcctgggcaggcaggacctctgtcccctctcagccggtccttggggctgcgtgtttctgtagaatgacgggtcaggctggccagaaccccaaaccttggccgtggggagtctgcgtggcggctctgccttgcccaggcatccttggtcctcactcgagttttcctaaggatgggatgagccccatgtgggactaaccttggctttacgacgtcaaagtttagatgagctggtgatatttttctcattatatccaaagtgtacctgttcgagtgaggacagttcttctgtctccaggatccctcctgggtggggattgtgcccgcctgggtctctgcccagattccagggctctccccgagccctgttcagaccatccgtgggggaggccttggcctcactcttacgtagataagtagcatggcgggttaatcattaactacaaggaacccctagtgatggagttggccactccctctctgcgcgctcgctcgctcactgaggccgggcgaccaaaggtcgcccgacgcccgggctttgcccgggcggcctcagtgagcgagcgagcgcgccagctggcgtaatagcgaagaggcccgcaccgatcgcccttcccaacagttgcgcagcctgaatggcgaatggcgattccgttgcaatggctggcggtaatattgttctggatattaccagcaaggccgatagtttgagttcttctactcaggcaagtgatgttattactaatcaaagaagtattgcgacaacggttaatttgcgtgatggacagactcttttactcggtggcctcactgattataaaaacacttctcaggattctggcgtaccgttcctgtctaaaatccctttaatcggcctcctgtttagctcccgctctgattctaacgaggaaagcacgttatacgtgctcgtcaaagcaaccatagtacgcgccctgtagcggcgcattaagcgcggcgggtgtggtggttacgcgcagcgtgaccgctacacttgccagcgccctagcgcccgctcctttcgctttcttcccttcctttctcgccacgttcgccggctttccccgtcaagctctaaatcgggggctccctttagggttccgatttagtgctttacggcacctcgaccccaaaaaacttgattagggtgatggttcacgtagtgggccatcgccctgatagacggtttttcgccctttgacgttggagtccacgttctttaatagtggactcttgttccaaactggaacaacactcaaccctatctcggtctattcttttgatttataagggattttgccgatttcggcctattggttaaaaaatgagctgatttaacaaaaatttaacgcgaattttaacaaaatattaacgtttacaatttaaatatttgcttatacaatcttcctgtttttggggcttttctgattatcaaccggggtacatatgattgacatgctagttttacgattaccgttcatcgattctcttgtttgctccagactctcaggcaatgacctgatagcctttgtagagacctctcaaaaatagctaccctctccggcatgaatttatcagctagaacggttgaatatcatattgatggtgatttgactgtctccggcctttctcacccgtttgaatctttacctacacattactcaggcattgcatttaaaatatatgagggttctaaaaatttttatccttgcgttgaaataaaggcttctcccgcaaaagtattacagggtcataatgtttttggtacaaccgatttagctttatgctctgaggctttattgcttaattttgctaattctttgccttgcctgtatgatttattggatgttggaatcgcctgatgcggtattttctccttacgcatctgtgcggtatttcacaccgcatatggtgcactctcagtacaatctgctctgatgccgcatagttaagccagccccgacacccgccaacacccgctgacgcgccctgacgggcttgtctgctcccggcatccgcttacagacaagctgtgaccgtctccgggagctgcatgtgtcagaggttttcaccgtcatcaccgaaacgcgcgagacgaaagggcctcgtgatacgcctatttttataggttaatgtcatgataataatggtttcttagacgtcaggtggcacttttcggggaaatgtgcgcggaacccctatttgtttatttttctaaatacattcaaatatgtatccgctcatgagacaataaccctgataaatgcttcaataatattgaaaaaggaagagtatgagtattcaacatttccgtgtcgcccttattcccttttttgcggcattttgccttcctgtttttgctcacccagaaacgctggtgaaagtaaaagatgctgaagatcagttgggtgcacgagtgggttacatcgaactggatctcaacagcggtaagatccttgagagttttcgccccgaagaacgttttccaatgatgagcacttttaaagttctgctatgtggcgcggtattatcccgtattgacgccgggcaagagcaactcggtcgccgcatacactattctcagaatgacttggttgagtactcaccagtcacagaaaagcatcttacggatggcatgacagtaagagaattatgcagtgctgccataaccatgagtgataacactgcggccaacttacttctgacaacgatcggaggaccgaaggagctaaccgcttttttgcacaacatgggggatcatgtaactcgccttgatcgttgggaaccggagctgaatgaagccataccaaacgacgagcgtgacaccacgatgcctgtagcaatggcaacaacgttgcgcaaactattaactggcgaactacttactctagcttcccggcaacaattaatagactggatggaggcggataaagttgcaggaccacttctgcgctcggcccttccggctggctggtttattgctgataaatctggagccggtgagcgtgggtctcgcggtatcattgcagcactggggccagatggtaagccctcccgtatcgtagttatctacacgacggggagtcaggcaactatggatgaacgaaatagacagatcgctgagataggtgcctcactgattaagcattggtaactgtcagaccaagtttactcatatatactttagattgatttaaaacttcatttttaatttaaaaggatctaggtgaagatcctttttgataatctcatgaccaaaatcccttaacgtgagttttcgttccactgagcgtcagaccccgtagaaaagatcaaaggatcttcttgagatcctttttttctgcgcgtaatctgctgcttgcaaacaaaaaaaccaccgctaccagcggtggtttgtttgccggatcaagagctaccaactctttttccgaaggtaactggcttcagcagagcgcagataccaaatactgtccttctagtgtagccgtagttaggccaccacttcaagaactctgtagcaccgcctacatacctcgctctgctaatcctgttaccagtggctgctgccagtggcgataagtcgtgtcttaccgggttggactcaagacgatagttaccggataaggcgcagcggtcgggctgaacggggggttcgtgcacacagcccagcttggagcgaacgacctacaccgaactgagatacctacagcgtgagctatgagaaagcgccacgcttcccgaagggagaaaggcggacaggtatccggtaagcggcagggtcggaacaggagagcgcacgagggagcttccagggggaaacgcctggtatctttatagtcctgtcgggtttcgccacctctgacttgagcgtcgatttttgtgatgctcgtcaggggggcggagcctatggaaaaacgccagcaacgcggcctttttacggttcctggccttttgctggccttttgctcacatgttctttcctgcgttatcccctgattctgtggataaccgtattaccgcctttgagtgagctgataccgctcgccgcagccgaacgaccgagcgcagcgagtcagtgagcgaggaagcggaagagcgcccaatacgcaaaccgcctctccccgcgcgttggccgattcattaatg

SEQ ID NO: 2 - DNA, 7413 bp, synthetic construct
  misc_feature 1..7413: note = Synthesized sequence pBW1490
  source 1..7413: mol_type = other DNA
cagctgcgcgctcgctcgctcactgaggccgcccgggcaaagcccgggcgtcgggcgacctttggtcgcccggcctcagtgagcgagcgagcgcgcagagagggagtggccaactccatcactaggggttccttgtagttaatgattaacccgccatgctacttatctacgtaatgggggaggagaagggcctgcccccacccggcagcctcaggaggggcagctcgggcgggatatggaaagaggccacagcagtgagcagagacacagaggaggaaggggccctgagctggggagacccccacggggtagggcgtgggggccacgggcccacctcctccccatctcctctgtctccctgtctctgtctctctctccctcccccaccctctccccagtcctaccccctcctcacccctcctcccccagcactgcctctgtcactctcgcccacgtggatgtggaggaagagggggcgggagcaaggggcgggcaccctcccttcaacctgacctgggacagtttcccttccgctcacctccgcctgagcagtggagaaggcggcactctggtggggctgctccaaatcatggcctcttggccaagattgatagcttgtgcctgtccctgagtcccagtccatcacgagcagctggtttctaagatgctatttcccgtataaagcatgagaccgtgacttgccagccccacagagccccgcccttgtccatcactggcatctggactccagcctgggttggggcaaagagggaaatgagatcatgtcctaaccctgatcctcttgtcccacagatatccagaaccctgaccctgccgtgtaccagctgagagactctaaatccagtgacaagtctgtctgcctatacgcgtaatgaaagaccccacctgtaggtttggcaagctaggatcaaggttaggaacagagagacagcagaatatgggccaaacaggatatctgtggtaagcagttcctgccccggctcagggccaagaacagttggaacagcagaatatgggccaaacaggatatctgtggtaagcagttcctgccccggctcagggccaagaacagatggtccccagatgcggtcccgccctcagcagtttctagagaaccatcagatgtttccagggtgccccaaggacctgaaatgaccctgtgccttatttgaactaaccaatcagttcgcttctcgcttctgttcgcgcgcttctgctccccgagctcaataaaagagcccacaacccctcactcggcgcgattcacctgcgcgtctacgccaccatggcactccccgtcaccgcccttctcttgcccctcgccctgctgctgcatgctgccaggcccgacattgtgctcactcagtcacctcccagcctggccatgagcctgggaaaaagggccaccatctcctgtagagccagtgagtccgtcacaatcttggggagccatcttattcactggtatcagcagaagcccgggcagcctccaacccttcttattcagctcgcgtcaaacgtccagacgggtgtacctgccagattttctggtagcgggtcccgcactgattttacactgaccatagatccagtggaagaagacgatgtggccgtgtattattgtctgcagagcagaacgattcctcgcacatttggtgggggtactaagctggagattaagggaagcacgtccggctcagggaagccgggctccggcgagggaagcacgaaggggcaaattcagctggtccagagcggacctgagctgaaaaaacccggcgagactgttaagatcagttgtaaagcatctggctataccttcaccgactacagcataaattgggtgaaacgggcccctggaaagggcctcaaatggatgggttggatcaataccgaaactagggagcctgcttatgcatatgacttccgcgggagattcgccttttcactcgagacatctgcctctactgcttacctccaaataaacaacctcaagtatgaagatacagccacttacttttgcgccctcgactatagttacgccatggactactggggacagggaacctccgttaccgtcagttccgcggccgcaaccacaacacctgctccaaggccccccacacccgctccaactatagccagccaaccattgagcctcagacctgaagcttgcaggcccgcagcaggaggcgccgtccatacgcgaggcctggacttcgcgtgtgatatttatatttgggcccctttggccggaacatgtggggtgttgcttctctcccttgtgatcactctgtattgtaagcgcgggagaaagaagctcctgtacatcttcaagcagccttttatgcgacctgtgcaaaccactcaggaagaagatgggtgttcatgccgcttccccgaggaggaagaaggagggtgtgaactgagggtgaaattttctagaagcgccgatgctcccgcatatcagcagggtcagaatcagctctacaatgaattgaatctcggcaggcgagaagagtacgatgttctggacaagagacggggcagggatcccgagatggggggaaagccccggagaaaaaatcctcaggaggggttgtacaatgagctgcagaaggacaagatggctgaagcctatagcgagatcggaatgaaaggcgaaagacgcagaggcaaggggcatgacggtctgtaccagggtctctctacagccaccaaggacacttatgatgcgttgcatatgcaagccttgccaccccgctaagcggccgcgctttatttgtgaaatttgtgatgctattgctttatttgtaaccattataagctgcaataaacaagttaacaacaacaattgcattcattttatgtttcaggttcagggggagatgtgggaggttttttaaagctcaccggttttgattctcaaacaaatgtgtcacaaagtaaggattctgatgtgtatatcacagacaaaactgtgctagacatgaggtctatggacttcaagagcaacagtgctgtggcctggagcaacaaatctgactttgcatgtgcaaacgccttcaacaacagcattattccagaagacaccttcttccccagcccaggtaagggcagctttggtgccttcgcaggctgtttccttgcttcaggaatggccaggttctgcccagagctctggtcaatgatgtctaaaactcctctgattggtggtaccggttctgggcggtgctacaactgggctggcggccaggatggttcttaggtaggtggggtcggcggtcaggtgtcccagagccaggggtctggagggaccttccaccctcagtccctggcaggtcggggggtgctgaggcgggcctggccctggcagcccaggggtcccggagcgaggggtctggagggacctttcactctcagtccctggcaggtcggggggtgctgtggcaggcccagccttggcccccagctctgccccttaccctgagctgtgtggctttgggcagctcgaactcctgggttcctctctgggccccaactcctcccctggcccaagtcccctctttgctcctgggcaggcaggacctctgtcccctctcagccggtccttggggctgcgtgtttctgtagtacgtagataagtagcatggcgggttaatcattaactacaaggaacccctagtgatggagttggccactccctctctgcgcgctcgctcgctcactgaggccgggcgaccaaaggtcgcccgacgcccgggctttgcccgggcggcctcagtgagcgagcgagcgcgccagctggcgtaatagcgaagaggcccgcaccgatcgcccttcccaacagttgcgcagcctgaatggcgaatggcgattccgttgcaatggctggcggtaatattgttctggatattaccagcaaggccgatagtttgagttcttctactcaggcaagtgatgttattactaatcaaagaagtattgcgacaacggttaatttgcgtgatggacagactcttttactcggtggcctcactgattataaaaacacttctcaggattctggcgtaccgttcctgtctaaaatccctttaatcggcctcctgtttagctcccgctctgattctaacgaggaaagcacgttatacgtgctcgtcaaagcaaccatagtacgcgccctgtagcggcgcattaagcgcggcgggtgtggtggttacgcgcagcgtgaccgctacacttgccagcgccctagcgcccgctcctttcgctttcttcccttcctttctcgccacgttcgccggctttccccgtcaagctctaaatcgggggctccctttagggttccgatttagtgctttacggcacctcgaccccaaaaaacttgattagggtgatggttcacgtagtgggccatcgccctgatagacggtttttcgccctttgacgttggagtccacgttctttaatagtggactcttgttccaaactggaacaacactcaaccctatctcggtctattcttttgatttataagggattttgccgatttcggcctattggttaaaaaatgagctgatttaacaaaaatttaacgcgaattttaacaaaatattaacgtttacaatttaaatatttgcttatacaatcttcctgtttttggggcttttctgattatcaaccggggtacatatgattgacatgctagttttacgattaccgttcatcgattctcttgtttgctccagactctcaggcaatgacctgatagcctttgtagagacctctcaaaaatagctaccctctccggcatgaatttatcagctagaacggttgaatatcatattgatggtgatttgactgtctccggcctttctcacccgtttgaatctttacctacacattactcaggcattgcatttaaaatatatgagggttctaaaaatttttatccttgcgttgaaataaaggcttctcccgcaaaagtattacagggtcataatgtttttggtacaaccgatttagctttatgctctgaggctttattgcttaattttgctaattctttgccttgcctgtatgatttattggatgttggaatcgcctgatgcggtattttctccttacgcatctgtgcggtatttcacaccgcatatggtgcactctcagtacaatctgctctgatgccgcatagttaagccagccccgacacccgccaacacccgctgacgcgccctgacgggcttgtctgctcccggcatccgcttacagacaagctgtgaccgtctccgggagctgcatgtgtcagaggttttcaccgtcatcaccgaaacgcgcgagacgaaagggcctcgtgatacgcctatttttataggttaatgtcatgataataatggtttcttagacgtcaggtggcacttttcggggaaatgtgcgcggaacccctatttgtttatttttctaaatacattcaaatatgtatccgctcatgagacaataaccctgataaatgcttcaataatattgaaaaaggaagagtatgagtattcaacatttccgtgtcgcccttattcccttttttgcggcattttgccttcctgtttttgctcacccagaaacgctggtgaaagtaaaagatgctgaagatcagttgggtgcacgagtgggttacatcgaactggatctcaacagcggtaagatccttgagagttttcgccccgaagaacgttttccaatgatgagcacttttaaagttctgctatgtggcgcggtattatcccgtattgacgccgggcaagagcaactcggtcgccgcatacactattctcagaatgacttggttgagtactcaccagtcacagaaaagcatcttacggatggcatgacagtaagagaattatgcagtgctgccataaccatgagtgataacactgcggccaacttacttctgacaacgatcggaggaccgaaggagctaaccgcttttttgcacaacatgggggatcatgtaactcgccttgatcgttgggaaccggagctgaatgaagccataccaaacgacgagcgtgacaccacgatgcctgtagcaatggcaacaacgttgcgcaaactattaactggcgaactacttactctagcttcccggcaacaattaatagactggatggaggcggataaagttgcaggaccacttctgcgctcggcccttccggctggctggtttattgctgataaatctggagccggtgagcgtgggtctcgcggtatcattgcagcactggggccagatggtaagccctcccgtatcgtagttatctacacgacggggagtcaggcaactatggatgaacgaaatagacagatcgctgagataggtgcctcactgattaagcattggtaactgtcagaccaagtttactcatatatactttagattgatttaaaacttcatttttaatttaaaaggatctaggtgaagatcctttttgataatctcatgaccaaaatcccttaacgtgagttttcgttccactgagcgtcagaccccgtagaaaagatcaaaggatcttcttgagatcctttttttctgcgcgtaatctgctgcttgcaaacaaaaaaaccaccgctaccagcggtggtttgtttgccggatcaagagctaccaactctttttccgaaggtaactggcttcagcagagcgcagataccaaatactgtccttctagtgtagccgtagttaggccaccacttcaagaactctgtagcaccgcctacatacctcgctctgctaatcctgttaccagtggctgctgccagtggcgataagtcgtgtcttaccgggttggactcaagacgatagttaccggataaggcgcagcggtcgggctgaacggggggttcgtgcacacagcccagcttggagcgaacgacctacaccgaactgagatacctacagcgtgagctatgagaaagcgccacgcttcccgaagggagaaaggcggacaggtatccggtaagcggcagggtcggaacaggagagcgcacgagggagcttccagggggaaacgcctggtatctttatagtcctgtcgggtttcgccacctctgacttgagcgtcgatttttgtgatgctcgtcaggggggcggagcctatggaaaaacgccagcaacgcggcctttttacggttcctggccttttgctggccttttgctcacatgttctttcctgcgttatcccctgattctgtggataaccgtattaccgcctttgagtgagctgataccgctcgccgcagccgaacgaccgagcgcagcgagtcagtgagcgaggaagcggaagagcgcccaatacgcaaaccgcctctccccgcgcgttggccgattcattaatg

SEQ ID NO: 3 - skipped

SEQ ID NO: 4 - protein, 5 aa, synthetic construct
  REGION 1..5: note = Exemplary linker sequence
DGGGS

SEQ ID NO: 5 - protein, 5 aa, synthetic construct
  REGION 1..5: note = Exemplary linker sequence
TGEKP

SEQ ID NO: 6 - protein, 4 aa, synthetic construct
  REGION 1..4: note = Exemplary linker sequence
GGRR

SEQ ID NO: 7 - protein, 5 aa, synthetic construct
  REGION 1..5: note = Exemplary linker sequence
GGGGS

SEQ ID NO: 8 - protein, 14 aa, synthetic construct
  REGION 1..14: note = Exemplary linker sequence
EGKSSGSGSESKVD

SEQ ID NO: 9 - protein, 18 aa, synthetic construct
  REGION 1..18: note = Exemplary linker sequence
KESGSVSSEQLAQFRSLD

SEQ ID NO: 10 - protein, 8 aa, synthetic construct
  REGION 1..8: note = Exemplary linker sequence
GGRRGGGS

SEQ ID NO: 11 - protein, 9 aa, synthetic construct
  REGION 1..9: note = Exemplary linker sequence
LRQRDGERP

SEQ ID NO: 12 - protein, 12 aa, synthetic construct
  REGION 1..12: note = Exemplary linker sequence
LRQKDGGGSERP

SEQ ID NO: 13 - protein, 16 aa, synthetic construct
  REGION 1..16: note = Exemplary linker sequence
LRQKDGGGSGGGSERP

SEQ ID NO: 14 - skipped

SEQ ID NO: 15 - protein, 7 aa, synthetic construct
  REGION 1..7: note = Cleavage sequence by TEV protease
ENLYFQG

SEQ ID NO: 16 - protein, 7 aa, synthetic construct
  REGION 1..7: note = Cleavage sequence by TEV protease
ENLYFQS

SEQ ID NO: 17 - protein, 22 aa, synthetic construct
  REGION 1..22: note = Self-cleaving polypeptide comprising 2A site
GSGATNFSLLKQAGDVEENPGP

SEQ ID NO: 18 - protein, 19 aa, synthetic construct
  REGION 1..19: note = Self-cleaving polypeptide comprising 2A site
ATNFSLLKQAGDVEENPGP

SEQ ID NO: 19 - protein, 14 aa, synthetic construct
  REGION 1..14: note = Self-cleaving polypeptide comprising 2A site
LLKQAGDVEENPGP

SEQ ID NO: 20 - protein, 21 aa, synthetic construct
  REGION 1..21: note = Self-cleaving polypeptide comprising 2A site
GSGEGRGSLLTCGDVEENPGP

SEQ ID NO: 21 - protein, 18 aa, synthetic construct
  REGION 1..18: note = Self-cleaving polypeptide comprising 2A site
EGRGSLLTCGDVEENPGP

SEQ ID NO: 22 - protein, 13 aa, synthetic construct
  REGION 1..13: note = Self-cleaving polypeptide comprising 2A site
LLTCGDVEENPGP

SEQ ID NO: 23 - protein, 23 aa, synthetic construct
  REGION 1..23: note = Self-cleaving polypeptide comprising 2A site
GSGQCTNYALLKLAGDVESNPGP

SEQ ID NO: 24 - protein, 20 aa, synthetic construct
  REGION 1..20: note = Self-cleaving polypeptide comprising 2A site
QCTNYALLKLAGDVESNPGP

SEQ ID NO: 25 - protein, 14 aa, synthetic construct
  REGION 1..14: note = Self-cleaving polypeptide comprising 2A site
LLKLAGDVESNPGP

SEQ ID NO: 26 - protein, 25 aa, synthetic construct
  REGION 1..25: note = Self-cleaving polypeptide comprising 2A site
GSGVKQTLNFDLLKLAGDVESNPGP

SEQ ID NO: 27 - protein, 22 aa, synthetic construct
  REGION 1..22: note = Self-cleaving polypeptide comprising 2A site
VKQTLNFDLLKLAGDVESNPGP

SEQ ID NO: 28 - protein, 14 aa, synthetic construct
  REGION 1..14: note = Self-cleaving polypeptide comprising 2A site
LLKLAGDVESNPGP

SEQ ID NO: 29 - protein, 19 aa, synthetic construct
  REGION 1..19: note = Self-cleaving polypeptide comprising 2A site
LLNFDLLKLAGDVESNPGP

SEQ ID NO: 30 - protein, 19 aa, synthetic construct
  REGION 1..19: note = Self-cleaving polypeptide comprising 2A site
TLNFDLLKLAGDVESNPGP

SEQ ID NO: 31 - protein, 14 aa, synthetic construct
  REGION 1..14: note = Self-cleaving polypeptide comprising 2A site
LLKLAGDVESNPGP

SEQ ID NO: 32 - protein, 17 aa, synthetic construct
  REGION 1..17: note = Self-cleaving polypeptide comprising 2A site
NFDLLKLAGDVESNPGP

SEQ ID NO: 33 - protein, 20 aa, synthetic construct
  REGION 1..20: note = Self-cleaving polypeptide comprising 2A site
QLLNFDLLKLAGDVESNPGP

SEQ ID NO: 34 - protein, 24 aa, synthetic construct
  REGION 1..24: note = Self-cleaving polypeptide comprising 2A site
APVKQTLNFDLLKLAGDVESNPGP

SEQ ID NO: 35 - protein, 40 aa, synthetic construct
  REGION 1..40: note = Self-cleaving polypeptide comprising 2A site
VTELLYRMKRAETYCPRPLLAIHPTEARHKQKIVAPVKQT

SEQ ID NO: 36 - protein, 18 aa, synthetic construct
  REGION 1..18: note = Self-cleaving polypeptide comprising 2A site
LNFDLLKLAGDVESNPGP

SEQ ID NO: 37 - protein, 40 aa, synthetic construct
  REGION 1..40: note = Self-cleaving polypeptide comprising 2A site
LLAIHPTEARHKQKIVAPVKQTLNFDLLKLAGDVESNPGP

SEQ ID NO: 38 - protein, 33 aa, synthetic construct
  REGION 1..33: note = Self-cleaving polypeptide comprising 2A site
EARHKQKIVAPVKQTLNFDLLKLAGDVESNPGP

SEQ ID NO: 39 - DNA, 10 bp, synthetic construct
  misc_feature 1..10: note = Consensus Kozak sequence
  source 1..10: mol_type = other DNA
gccrccatgg

SEQ ID NO: 40 - protein, 9 aa, synthetic construct
  REGION 1..9: note = Motif
LAGLIDADG